European Patent Application EP 4 201 430 A1, published June 28, 2023. Title: Modified antibody for site-specific conjugation and its diagnostic use. Applicant: Roche Diagnostics GmbH F. Hoffmann-La Roche AG. The sequence listing filed with the application follows.

SEQUENCE LISTING (29 sequences)

SEQ ID NO: 1 - protein, 329 aa, Homo sapiens
ASTKGPSVFPLAPSSKSTSGGTAALGCLVKDYFPEPVTVSWNSGALTSGVHTFPAVLQSSGLYSLSSVVTVPSSSLGTQTYICNVNHKPSNTKVDKKVEPKSCDKTHTCPPCPAPELLGGPSVFLFPPKPKDTLMISRTPEVTCVVVDVSHEDPEVKFNWYVDGVEVHNAKTKPREEQYNSTYRVVSVLTVLHQDWLNGKEYKCKVSNKALPAPIEKTISKAKGQPREPQVYTLPPSRDELTKNQVSLTCLVKGFYPSDIAVEWESNGQPENNYKTTPPVLDSDGSFFLYSKLTVDKSRWQQGNVFSCSVMHEALHNHYTQKSLSLSPG

SEQ ID NO: 2 - protein, 325 aa, Homo sapiens
ASTKGPSVFPLAPCSRSTSESTAALGCLVKDYFPEPVTVSWNSGALTSGVHTFPAVLQSSGLYSLSSVVTVPSSNFGTQTYTCNVDHKPSNTKVDKTVERKCCVECPPCPAPPVAGPSVFLFPPKPKDTLMISRTPEVTCVVVDVSHEDPEVQFNWYVDGVEVHNAKTKPREEQFNSTFRVVSVLTVVHQDWLNGKEYKCKVSNKGLPAPIEKTISKTKGQPREPQVYTLPPSREEMTKNQVSLTCLVKGFYPSDIAVEWESNGQPENNYKTTPPMLDSDGSFFLYSKLTVDKSRWQQGNVFSCSVMHEALHNHYTQKSLSLSPG

SEQ ID NO: 3 - protein, 326 aa, Homo sapiens
ASTKGPSVFPLAPCSRSTSESTAALGCLVKDYFPEPVTVSWNSGALTSGVHTFPAVLQSSGLYSLSSVVTVPSSSLGTKTYTCNVDHKPSNTKVDKRVSPNMVPHAHHAQAPEFLGGPSVFLFPPKPKDTLMISRTPEVTCVVVDVSQEDPEVQFNWYVDGVEVHNAKTKPREEQFNSTYRVVSVLTVLHQDWLNGKEYKCKVSNKGLPSSIEKTISKAKGQPREPQVYTLPPSQEEMTKNQVSLTCLVKGFYPSDIAVEWESNGQPENNYKTTPPVLDSDGSFFLYSRLTVDKSRWQEGNVFSCSVMHEALHNHYTQKSLSLSLG

SEQ ID NO: 4 - protein, 326 aa, Homo sapiens; identical to SEQ ID NO: 3

SEQ ID NO: 5 - protein, 323 aa, Mus musculus
AKTTPPSVYPLAPGSAAQTNSMVTLGCLVKGYFPEPVTVTWNSGSLSSGVHTFPAVLQSDLYTLSSSVTVPSSTWPSETVTCNVAHPASSTKVDKKIVPRDCGCKPCICTVPEVSSVFIFPPKPKDVLTITLTPKVTCVVVDISKDDPEVQFSWFVDDVEVHTAQTQPREEQFNSTFRSVSELPIMHQDWLNGKEFKCRVNSAAFPAPIEKTISKTKGRPKAPQVYTIPPPKEQMAKDKVSLTCMITDFFPEDITVEWQWNGQPAENYKNTQPIMDTDGSYFVYSKLNVQKSNWEAGNTFTCSVLHEGLHNHHTEKSLSHSPG

SEQ ID NO: 6 - protein, 329 aa, Mus musculus
AKTTAPSVYPLAPVCGDTTGSSVTLGCLVKGYFPEPVTLTWNSGSLSSGVHTFPAVLQSDLYTLSSSVTVTSSTWPSQSITCNVAHPASSTKVDKKIEPRGPTIKPCPPCKCPAPNLLGGPSVFIFPPKIKDVLMISLSPIVTCVVVDVSEDDPDVQISWFVNNVEVHTAQTQTHREDYNSTLRVVSALPIQHQDWMSGKEFKCKVNNKDLPAPIERTISKPKGSVRAPQVYVLPPPEEEMTKKQVTLTCMVTDFMPEDIYVEWTNNGKTELNYKNTEPVLDSDGSYFMYSKLRVEKKNWVERNSYSCSVVHEGLHNHHTTKSFSRTPG

SEQ ID NO: 7 - protein, 335 aa, Mus musculus
AKTTPPSVYPLAPGCGDTTGSSVTLGCLVKGYFPESVTVTWNSGSLSSSVHTFPALLQSGLYTMSSSVTVPSSTWPSQTVTCSVAHPASSTTVDKKLEPSGPISTINPCPPCKECHKCPAPNLEGGPSVFIFPPNIKDVLMISLTPKVTCVVVDVSEDDPDVRISWFVNNVEVHTAQTQTHREDYNSTIRVVSALPIQHQDWMSGKEFKCKVNNKDLPSPIERTISKIKGLVRAPQVYILPPPAEQLSRKDVSLTCLVVGFNPGDISVEWTSNGHTEENYKDTAPVLDSDGSYFIYSKLDIKTSKWEKTDSFSCNVRHEGLKNYYLKKTISRSPG

SEQ ID NO: 8 - protein, 322 aa, Oryctolagus cuniculus
GQPKAPSVFPLAPCCGDTPSSTVTLGCLVKGYLPEPVTVTWNSGTLTNGVRTFPSVRQSSGLYSLSSVVSVTSSSQPVTCNVAHPATNTKVDKTVAPSTCSKPTCPPPELLGGPSVFIFPPKPKDTLMISRTPEVTCVVVDVSQDDPEVQFTWYINNEQVRTARPPLREQQFNSTIRVVSTLPIAHQDWLRGKEFKCKVHNKALPAPIEKTISKARGQPLEPKVYTMGPPREELSSRSVSLTCMINGFYPSDISVEWEKNGKAEDNYKTTPAVLDSDGSYFLYNKLSVPTSEWQRGDVFTCSVMHEALHNHYTQKSISRSPG

SEQ ID NO: 9 - protein, 330 aa, Ovis aries
ASTTPPKVYPLTSCCGDTSSSIVTLGCLVSSYMPEPVTVTWNSGALTSGVHTFPAILQSSGLYSLSSVVTVPASTSGAQTFICNVAHPASSTKVDKRVEPGCPDPCKHCRCPPPELPGGPSVFIFPPKPKDTLTISGTPEVTCVVVDVGQDDPEVQFSWFVDNVEVRTARTKPREEQFNSTFRVVSALPIQHQDWTGGKEFKCKVHNEGLPAPIVRTISRTKGQAREPQVYVLAPPQEELSKSTLSVTCLVTGFYPDYIAVEWQKNGQPESEDKYGTTTSQLDADGSYFLYSRLRVDKNSWQEGDTYACVVMHEALHNHYTQKSISKPPG

SEQ ID NO: 10 - protein, 106 aa, Homo sapiens
TVAAPSVFIFPPSDEQLKSGTASVVCLLNNFYPREAKVQWKVDNALQSGNSQESVTEQDSKDSTYSLSSTLTLSKADYEKHKVYACEVTHQGLSSPVTKSFNRGEC

SEQ ID NO: 11 - protein, 106 aa, Mus musculus
ADAAPTVSIFPPSSEQLTSGGASVVCFLNNFYPKDINVKWKIDGSERQNGVLNSWTDQDSKDSTYSMSSTLTLTKDEYERHNSYTCEATHKTSTSPIVKSFNRNEC

SEQ ID NO: 12 - protein, 103 aa, Oryctolagus cuniculus
DPVAPTVLIFPPAADQVATGTVTIVCVANKYFPDVTVTWEVDGTTQTTGIENSKTPQNSADCTYNLSSTLTLTSTQYNSHKEYTCKVTQGTTSVVQSFNRGDC

SEQ ID NO: 13 - protein, 104 aa, Ovis aries
PKSAPSVTLFPPSTEELSTNKATVVCLINDFYPGSVNVVWKADGSTINQNVKTTQASKQSNSKYAASSYLTLTGSEWKSKSSYTCEVTHEGSTVTKTVKPSECS

SEQ ID NO: 14 - protein, 5 aa, Artificial Sequence
  Q-tag
YRYRQ

SEQ ID NO: 15 - protein, 5 aa, Artificial Sequence
  Q-tag
RVRQR

SEQ ID NO: 16 - protein, 5 aa, Artificial Sequence
  Q-tag
YRQRT

SEQ ID NO: 17 - protein, 5 aa, Artificial Sequence
  Q-tag
RYGQR

SEQ ID NO: 18 - protein, 5 aa, Artificial Sequence
  Q-tag
RWRQR

SEQ ID NO: 19 - protein, 5 aa, Artificial Sequence
  Q-tag
IRQRQ

SEQ ID NO: 20 - protein, 5 aa, Artificial Sequence
  Q-tag
FRYRQ

SEQ ID NO: 21 - protein, 5 aa, Artificial Sequence
  K-tag
RYESK

SEQ ID NO: 22 - protein, 4 aa, Artificial Sequence
  Linker
GGGS

SEQ ID NO: 23 - protein, 4 aa, Artificial Sequence
  Linker
GGGP

SEQ ID NO: 24 - protein, 4 aa, Artificial Sequence
  Linker
ESGS

SEQ ID NO: 25 - protein, 4 aa, Artificial Sequence
  Linker
APAP

SEQ ID NO: 26 - protein, 18 aa, Artificial Sequence
  Linker
KESGSVSSEQLAQFRSLD

SEQ ID NO: 27 - protein, 14 aa, Artificial Sequence
  Linker
EGKSSGSGSESKST

SEQ ID NO: 28 - protein, 13 aa, Artificial Sequence
  Q-tag motif with two flexible linkers
GGGSYRYRQGGGS

SEQ ID NO: 29 - protein, 13 aa, Artificial Sequence
  Q-tag motif with two flexible linkers
GGGSRVRQRGGGS